European Patent Application EP 4 591 885 A2, published July 30, 2025. Title: ANTI-IL-6 ANTIBODY FORMULATION. Applicant: Novo Nordisk A/S. Application US PCT/US2020/030865, filed April 30, 2020. The sequence listing filed with the application follows.

SEQUENCE LISTING (10 sequences)

SEQ ID NO: 1 - protein, 5 aa, synthetic construct
  REGION 1..5: note = source = /note="Description of Artificial Sequence: Synthetic peptide"
SNYMI

SEQ ID NO: 2 - protein, 17 aa, synthetic construct
  REGION 1..17: note = source = /note="Description of Artificial Sequence: Synthetic peptide"
DLYYYAGDTYYADSVKG

SEQ ID NO: 3 - protein, 11 aa, synthetic construct
  REGION 1..11: note = source = /note="Description of Artificial Sequence: Synthetic peptide"
WADDHPPWIDL

SEQ ID NO: 4 - protein, 11 aa, synthetic construct
  REGION 1..11: note = source = /note="Description of Artificial Sequence: Synthetic peptide"
RASQGISSWLA

SEQ ID NO: 5 - protein, 7 aa, synthetic construct
  REGION 1..7: note = source = /note="Description of Artificial Sequence: Synthetic peptide"
KASTLES

SEQ ID NO: 6 - protein, 8 aa, synthetic construct
  REGION 1..8: note = source = /note="Description of Artificial Sequence: Synthetic peptide"
QQSWLGGS

SEQ ID NO: 7 - protein, 120 aa, synthetic construct
  REGION 1..120: note = source = /note="Description of Artificial Sequence: Synthetic polypeptide"
EVQLVESGGGLVQPGGSLRLSCAASGFTISSNYMIWVRQAPGKGLEWVSDLYYYAGDTYYADSVKGRFTMSRDISKNTVYLQMNSLRAEDTAVYYCARWADDHPPWIDLWGRGTLVTVSS

SEQ ID NO: 8 - protein, 106 aa, synthetic construct
  REGION 1..106: note = source = /note="Description of Artificial Sequence: Synthetic polypeptide"
DIQMTQSPSTLSASVGDRVTITCRASQGISSWLAWYQQKPGKAPKVLIYKASTLESGVPSRFSGSGSGTEFTLTISSLQPDDFATYYCQQSWLGGSFGQGTKLEIK

SEQ ID NO: 9 - protein, 450 aa, synthetic construct
  REGION 1..450: note = source = /note="Description of Artificial Sequence: Synthetic polypeptide"
EVQLVESGGGLVQPGGSLRLSCAASGFTISSNYMIWVRQAPGKGLEWVSDLYYYAGDTYYADSVKGRFTMSRDISKNTVYLQMNSLRAEDTAVYYCARWADDHPPWIDLWGRGTLVTVSSASTKGPSVFPLAPSSKSTSGGTAALGCLVKDYFPEPVTVSWNSGALTSGVHTFPAVLQSSGLYSLSSVVTVPSSSLGTQTYICNVNHKPSNTKVDKRVEPKSCDKTHTCPPCPAPELLGGPSVFLFPPKPKDTLYITREPEVTCVVVDVSHEDPEVKFNWYVDGVEVHNAKTKPREEQYNSTYRVVSVLTVLHQDWLNGKEYKCKVSNKALPAPIEKTISKAKGQPREPQVYTLPPSREEMTKNQVSLTCLVKGFYPSDIAVEWESNGQPENNYKTTPPVLDSDGSFFLYSKLTVDKSRWQQGNVFSCSVMHEALHNHYTQKSLSLSPGK

SEQ ID NO: 10 - protein, 213 aa, synthetic construct
  REGION 1..213: note = source = /note="Description of Artificial Sequence: Synthetic polypeptide"
DIQMTQSPSTLSASVGDRVTITCRASQGISSWLAWYQQKPGKAPKVLIYKASTLESGVPSRFSGSGSGTEFTLTISSLQPDDFATYYCQQSWLGGSFGQGTKLEIKRTVAAPSVFIFPPSDEQLKSGTASVVCLLNNFYPREAKVQWKVDNALQSGNSQESVTEQDSKDSTYSLSSTLTLSKADYEKHKVYACEVTHQGLSSPVTKSFNRGEC